European Patent Specification EP 4 110 958 B1, published September 10, 2025. Title: PRIMER SET OF FOOD POISONING BACTERIA USING NEXT GENERATION SEQUENCING AND DETECTION METHOD USING THEREOF. Applicant: Sanigen Co.,Ltd. KOREA FOOD & DRUG ADMINISTRATION. The sequence listing filed with the application follows.

SEQUENCE LISTING (78 sequences)

SEQ ID NO: 1 - DNA, 20 bp, Artificial Sequence
  1-F primer
gcgctcttctaaagtctcac

SEQ ID NO: 2 - DNA, 20 bp, Artificial Sequence
  1-R primer
cgaaattagcccagtagcac

SEQ ID NO: 3 - DNA, 21 bp, Artificial Sequence
  2-F primer
gaactgctggtacaacacctg

SEQ ID NO: 4 - DNA, 21 bp, Artificial Sequence
  2-R primer
tctgcactaatgaactgaccg

SEQ ID NO: 5 - DNA, 23 bp, Artificial Sequence
  3-F primer
ccgcttttggacctcaatctcgc

SEQ ID NO: 6 - DNA, 24 bp, Artificial Sequence
  3-R primer
gccttgtgcgcgttctttattgcc

SEQ ID NO: 7 - DNA, 21 bp, Artificial Sequence
  4-F primer
gcaagaattacctttggttga

SEQ ID NO: 8 - DNA, 21 bp, Artificial Sequence
  4-R primer
cctccatttgcttgtattcat

SEQ ID NO: 9 - DNA, 21 bp, Artificial Sequence
  5-F primer
cctacgacttgtttgatttgg

SEQ ID NO: 10 - DNA, 21 bp, Artificial Sequence
  5-R primer
ccacagaatgacctccattag

SEQ ID NO: 11 - DNA, 20 bp, Artificial Sequence
  6-F primer
tggagttgttgtggggcttc

SEQ ID NO: 12 - DNA, 20 bp, Artificial Sequence
  6-R primer
tgatgcgttcttttgcaccc

SEQ ID NO: 13 - DNA, 21 bp, Artificial Sequence
  7-F primer
ttatggcgagggacttggagc

SEQ ID NO: 14 - DNA, 21 bp, Artificial Sequence
  7-R primer
agaataatgcgccgttggacg

SEQ ID NO: 15 - DNA, 21 bp, Artificial Sequence
  8-F primer
atgttactgccgttgatagcg

SEQ ID NO: 16 - DNA, 22 bp, Artificial Sequence
  8-R primer
gctgcataatcccaatcatccc

SEQ ID NO: 17 - DNA, 22 bp, Artificial Sequence
  9-F primer
ggcgttcttctaactcataccc

SEQ ID NO: 18 - DNA, 22 bp, Artificial Sequence
  9-R primer
ctccatcacctaaggactgttc

SEQ ID NO: 19 - DNA, 21 bp, Artificial Sequence
  10-F primer
gccttattgtcttattggtct

SEQ ID NO: 20 - DNA, 21 bp, Artificial Sequence
  10-R primer
gaaaaatggaatagcacctaa

SEQ ID NO: 21 - DNA, 21 bp, Artificial Sequence
  11-F primer
gatgctgacgattctgtatta

SEQ ID NO: 22 - DNA, 21 bp, Artificial Sequence
  11-R primer
ataagtccttctcgattgtgt

SEQ ID NO: 23 - DNA, 21 bp, Artificial Sequence
  12-F primer
gatagatccagaggaagggcg

SEQ ID NO: 24 - DNA, 21 bp, Artificial Sequence
  12-R primer
tacgactgatccctgcaacac

SEQ ID NO: 25 - DNA, 21 bp, Artificial Sequence
  13-F primer
actgtctgaaactgctcctgt

SEQ ID NO: 26 - DNA, 21 bp, Artificial Sequence
  13-R primer
ggttgactctcttcattcacg

SEQ ID NO: 27 - DNA, 23 bp, Artificial Sequence
  14-F primer
ctcaggatgctaaaccagtagag

SEQ ID NO: 28 - DNA, 22 bp, Artificial Sequence
  14-R primer
ccggtacaagcaggattacaac

SEQ ID NO: 29 - DNA, 21 bp, Artificial Sequence
  15-F primer
tagtggattggactcaacgat

SEQ ID NO: 30 - DNA, 21 bp, Artificial Sequence
  15-R primer
tattaacaccgtagcctttcg

SEQ ID NO: 31 - DNA, 23 bp, Artificial Sequence
  16-F primer
acgagtcaacttttagcgaaggg

SEQ ID NO: 32 - DNA, 24 bp, Artificial Sequence
  16-R primer
ctctatttccaatcgcgtcagaac

SEQ ID NO: 33 - DNA, 20 bp, Artificial Sequence
  17-F primer
tcctgcttagatgatggagg

SEQ ID NO: 34 - DNA, 20 bp, Artificial Sequence
  17-R primer
ccaaaaggaagtgtctgctc

SEQ ID NO: 35 - DNA, 21 bp, Artificial Sequence
  18-F primer
tgacggatatgtttccacttc

SEQ ID NO: 36 - DNA, 21 bp, Artificial Sequence
  18-R primer
gtattccacctaacgcagaaa

SEQ ID NO: 37 - DNA, 21 bp, Artificial Sequence
  19-F primer
ctggtgatactctttggggta

SEQ ID NO: 38 - DNA, 22 bp, Artificial Sequence
  19-R primer
agccgttagattcggttgtttc

SEQ ID NO: 39 - DNA, 21 bp, Artificial Sequence
  20-F primer
gtgacgaagtagaagttatcg

SEQ ID NO: 40 - DNA, 21 bp, Artificial Sequence
  20-R primer
agttagtgtgtggagtaatcg

SEQ ID NO: 41 - DNA, 21 bp, Artificial Sequence
  21-F primer
ttgatggtgctgttgcggttc

SEQ ID NO: 42 - DNA, 19 bp, Artificial Sequence
  21-R primer
tgggagttggattgggtgc

SEQ ID NO: 43 - DNA, 21 bp, Artificial Sequence
  22-F primer
cgcactgaatatcgtactgga

SEQ ID NO: 44 - DNA, 20 bp, Artificial Sequence
  22-R primer
cgataatttcaccggcatcg

SEQ ID NO: 45 - DNA, 21 bp, Artificial Sequence
  23-F primer
gctgagtaaccaacaagataa

SEQ ID NO: 46 - DNA, 21 bp, Artificial Sequence
  23-R primer
agtaaacgctgttcataggtc

SEQ ID NO: 47 - DNA, 21 bp, Artificial Sequence
  24-F primer
gcagcttgcttacttactgct

SEQ ID NO: 48 - DNA, 21 bp, Artificial Sequence
  24-R primer
tacctgtaatctcgccatcat

SEQ ID NO: 49 - DNA, 21 bp, Artificial Sequence
  25-F primer
attcattgccctaacgtggac

SEQ ID NO: 50 - DNA, 25 bp, Artificial Sequence
  25-R primer
gctgtaaaaattgatcgtgactctc

SEQ ID NO: 51 - DNA, 20 bp, Artificial Sequence
  26-F primer
gtatggtggtgtaactgagc

SEQ ID NO: 52 - DNA, 20 bp, Artificial Sequence
  26-R primer
ccgtttcataaggcgagttg

SEQ ID NO: 53 - DNA, 21 bp, Artificial Sequence
  27-F primer
ctgctatttttcatccaaaga

SEQ ID NO: 54 - DNA, 21 bp, Artificial Sequence
  27-R primer
ttcttatcagtttgcacttca

SEQ ID NO: 55 - DNA, 20 bp, Artificial Sequence
  28-F primer
tgtcactccacacgaaggta

SEQ ID NO: 56 - DNA, 20 bp, Artificial Sequence
  28-R primer
tgcaaatagcgccttgcttg

SEQ ID NO: 57 - DNA, 21 bp, Artificial Sequence
  29-F primer
gccaagaggacagagtgagta

SEQ ID NO: 58 - DNA, 20 bp, Artificial Sequence
  29-R primer
atgaggactgtatgccccta

SEQ ID NO: 59 - DNA, 21 bp, Artificial Sequence
  30-F primer
taagaccaacagcaaccgccc

SEQ ID NO: 60 - DNA, 23 bp, Artificial Sequence
  30-R primer
actcgactggcgtaaccaaaagg

SEQ ID NO: 61 - DNA, 21 bp, Artificial Sequence
  31-F primer
gtttgtatgtgcgagcgggtg

SEQ ID NO: 62 - DNA, 21 bp, Artificial Sequence
  31-R primer
gtgaatgtcagcgccaccaac

SEQ ID NO: 63 - DNA, 21 bp, Artificial Sequence
  32-F primer
gcactgtctcatttcccagag

SEQ ID NO: 64 - DNA, 21 bp, Artificial Sequence
  32-R primer
cgcttcttggtcagaaaccag

SEQ ID NO: 65 - DNA, 19 bp, Artificial Sequence
  33-F primer
acctgtggcttctgctgtg

SEQ ID NO: 66 - DNA, 21 bp, Artificial Sequence
  33-R primer
ccagttgttgatttgcgggtg

SEQ ID NO: 67 - DNA, 22 bp, Artificial Sequence
  34-F primer
tccatctgtcccttttcctgcc

SEQ ID NO: 68 - DNA, 25 bp, Artificial Sequence
  34-R primer
cagccatttagtacctgacgttgtg

SEQ ID NO: 69 - DNA, 21 bp, Artificial Sequence
  35-F primer
gcgagcgatccttgtttggac

SEQ ID NO: 70 - DNA, 21 bp, Artificial Sequence
  35-R primer
gcggtgagttgctgttgttgg

SEQ ID NO: 71 - DNA, 20 bp, Artificial Sequence
  36-F primer
ctctgcctagatgtttatgg

SEQ ID NO: 72 - DNA, 21 bp, Artificial Sequence
  36-R primer
caataccatttctgtgctaag

SEQ ID NO: 73 - DNA, 21 bp, Artificial Sequence
  37-F primer
agcacatctctattccttctc

SEQ ID NO: 74 - DNA, 20 bp, Artificial Sequence
  37-R primer
tagcgttgcttcttcagtaa

SEQ ID NO: 75 - DNA, 21 bp, Artificial Sequence
  38-F primer
tggggccatctttccgcatta

SEQ ID NO: 76 - DNA, 21 bp, Artificial Sequence
  38-R primer
taccctgcaccaagcatccaa

SEQ ID NO: 77 - DNA, 21 bp, Artificial Sequence
  39-F primer
aacggggcatctggttctctc

SEQ ID NO: 78 - DNA, 21 bp, Artificial Sequence
  39-R primer
tggtggtgtcaggaaagggac